European Patent Application EP 4 574 164 A1, published June 25, 2025. Title: COMBINATIONS. Applicant: Universität Bern. Application EP. The sequence listing filed with the application follows.

SEQUENCE LISTING (24 sequences)

SEQ ID NO: 1 - DNA, 345 bp, Homo sapiens
  source 1..345: mol_type = genomic DNA
caagccaaacacaaacagcggaaacgccttaagtccagctgtaagagacaccctttgtacgtggacttcagtgacgtggggtggaatgactggattgtggctcccccggggtatcacgccttttactgccacggagaatgcccttttcctctggctgatcatctgaactccactaatcatgccattgttcagacgttggtcaactctgttaactctaagattcctaaggcatgctgtgtcccgacagaactcagtgctatctcgatgctgtaccttgacgagaatgaaaaggttgtattaaagaactatcaggacatggttgtggagggttgtgggtgtcgctag

SEQ ID NO: 2 - DNA, 351 bp, Homo sapiens
  source 1..351: mol_type = genomic DNA
agccctaagcatcactcacagcgggccaggaagaagaataagaactgccggcgccactcgctctatgtggacttcagcgatgtgggctggaatgactggattgtggccccaccaggctaccaggccttctactgccatggggactgcccctttccactggctgaccacctcaactcaaccaaccatgccattgtgcagaccctggtcaattctgtcaattccagtatccccaaagcctgttgtgtgcccactgaactgagtgccatctccatgctgtacctggatgagtatgataaggtggtactgaaaaattatcaggagatggtagtagagggatgtgggtgccgctga

SEQ ID NO: 3 - DNA, 399 bp, Homo sapiens
  source 1..399: mol_type = genomic DNA
aatcaaaaccgcaataaatccagctctcatcaggactcctccagaatgtccagtgttggagattataacacaagtgagcaaaaacaagcctgtaagaagcacgaactctatgtgagcttccgggatctgggatggcaggactggattatagcaccagaaggatacgctgcattttattgtgatggagaatgttcttttccacttaacgcccatatgaatgccaccaaccacgctatagttcagactctggttcatctgatgtttcctgaccacgtaccaaagccttgttgtgctccaaccaaattaaatgccatctctgttctgtactttgatgacagctccaatgtcattttgaaaaaatatagaaatatggtagtacgctcatgtggctgccactaa

SEQ ID NO: 4 - DNA, 399 bp, Homo sapiens
  source 1..399: mol_type = genomic DNA
caacagagtcgtaatcgctctacccagtcccaggacgtggcgcgggtctccagtgcttcagattacaacagcagtgaattgaaaacagcctgcaggaagcatgagctgtatgtgagtttccaagacctgggatggcaggactggatcattgcacccaagggctatgctgccaattactgtgatggagaatgctccttcccactcaacgcacacatgaatgcaaccaaccacgcgattgtgcagaccttggttcaccttatgaaccccgagtatgtccccaaaccgtgctgtgcgccaactaagctaaatgccatctcggttctttactttgatgacaactccaatgtcattctgaaaaaatacaggaatatggttgtaagagcttgtggatgccactaa

SEQ ID NO: 5 - DNA, 420 bp, Homo sapiens
  source 1..420: mol_type = genomic DNA
tccacggggagcaaacagcgcagccagaaccgctccaagacgcccaagaaccaggaagccctgcggatggccaacgtggcagagaacagcagcagcgaccagaggcaggcctgtaagaagcacgagctgtatgtcagcttccgagacctgggctggcaggactggatcatcgcgcctgaaggctacgccgcctactactgtgagggggagtgtgccttccctctgaactcctacatgaacgccaccaaccacgccatcgtgcagacgctggtccacttcatcaacccggaaacggtgcccaagccctgctgtgcgcccacgcagctcaatgccatctccgtcctctacttcgatgacagctccaacgtcatcctgaagaaatacagaaacatggtggtccgggcctgtggctgccactag

SEQ ID NO: 6 - DNA, 420 bp, Homo sapiens
  source 1..420: mol_type = genomic DNA
gcagtgaggccactgaggaggaggcagccgaagaaaagcaacgagctgccgcaggccaaccgactcccagggatctttgatgacgtccacggctcccacggccggcaggtctgccgtcggcacgagctctacgtcagcttccaggacctcggctggctggactgggtcatcgctccccaaggctactcggcctattactgtgagggggagtgctccttcccactggactcctgcatgaatgccaccaaccacgccatcctgcagtccctggtgcacctgatgaagccaaacgcagtccccaaggcgtgctgtgcacccaccaagctgagcgccacctctgtgctctactatgacagcagcaacaacgtcatcctgcgcaagcaccgcaacatggtggtcaaggcctgcggctgccactga

SEQ ID NO: 7 - DNA, 363 bp, Homo sapiens
  source 1..363: mol_type = genomic DNA
gccccactggccactcgccagggcaagcgacccagcaagaaccttaaggctcgctgcagtcggaaggcactgcatgtcaacttcaaggacatgggctgggacgactggatcatcgcaccccttgagtacgaggctttccactgcgaggggctgtgcgagttcccattgcgctcccacctggagcccacgaatcatgcagtcatccagaccctgatgaactccatggaccccgagtccacaccacccacctgctgtgtgcccacgcggctgagtcccatcagcatcctcttcattgactctgccaacaacgtggtgtataagcagtatgaggacatggtcgtggagtcgtgtggctgcaggtag

SEQ ID NO: 8 - DNA, 360 bp, Mus musculus
  source 1..360: mol_type = genomic DNA
accgccttcgccagccgtcacggcaagcgacatggcaagaagtccaggctgcgctgcagcagaaagcctctgcacgtgaattttaaggagttaggctgggacgactggattatcgcgcccctagagtacgaggcctatcactgcgagggcgtgtgcgactttccgctgcgctcgcaccttgagcccactaaccatgccatcattcagacgctgatgaactccatggacccgggctccaccccgcctagctgctgcgttcccaccaaactgactcccattagcatcctgtacatcgacgcgggcaataatgtagtctacaagcagtatgaggacatggtggtggagtcctgcggctgtagg

SEQ ID NO: 9 - DNA, 438 bp, Mus musculus
  source 1..438: mol_type = genomic DNA
actgcgctggctgggactcggggagcgcagggaagcggtggtggcggcggtggcggtggcggcggcggcggcggcggcggcggcggcggcggcggcgcaggcaggggccacgggcgcagaggccggagccgctgcagtcgcaagtcactgcacgtggactttaaggagctgggctgggacgactggatcatcgcgccattagactacgaggcataccactgcgagggcgtttgcgactttcctctgcgctcgcacctggagcctaccaaccacgccatcattcagacgctgctcaactccatggcgcccgacgctgcgccagcctcctgctgcgtgcccgcaaggctcagtcccatcagcattctctacatcgatgccgccaacaacgtggtctacaagcagtacgaagacatggtggtggaggcctgcggctgcagg

SEQ ID NO: 10 - DNA, 327 bp, Homo sapiens
  source 1..327: mol_type = genomic DNA
aacgccaaaggaaactactgtaagaggaccccgctctacatcgacttcaaggagattgggtgggactcctggatcatcgctccgcctggatacgaagcctatgaatgccgtggtgtttgtaactaccccctggcagagcatctcacacccacaaagcatgcaattatccaggccttggtccacctcaagaattcccagaaagcttccaaagcctgctgtgtgcccacaaagctagagcccatctccatcctctatttagacaaaggcgtcgtcacctacaagtttaaatacgaaggcatggccgtctccgaatgtggctgtagatag

SEQ ID NO: 11 - DNA, 333 bp, Homo sapiens
  source 1..333: mol_type = genomic DNA
agcgccggggctggcagccactgtcaaaagacctccctgcgggtaaacttcgaggacatcggctgggacagctggatcattgcacccaaggagtatgaagcctacgagtgtaagggcggctgcttcttccccttggctgacgatgtgacgccgacgaaacacgctatcgtgcagaccctggtgcatctcaagttccccacaaaggtgggcaaggcctgctgtgtgcccaccaaactgagccccatctccgtcctctacaaggatgacatgggggtgcccaccctcaagtaccattacgagggcatgagcgtggcagagtgtgggtgcaggtag

SEQ ID NO: 12 - DNA, 3545 bp, synthetic construct
  source 1..3545: mol_type = other DNA; note = L51P
gccgccgccgccgtcgccgccgccggagtcctcgccccgccgcgctgcgcccggctcgcgctgcgctagtcgctccgcttcccacaccccgccggggactggcagccgccgccgcacatctgccgccacagcctccgccggctacccgaacgttctcggggccagcgccgagtggatcaccggggaccgcgaggcacccgcgcgccgcagaccccgcgcgggctggagcacccggcagagcgcgccacagcgccgtggcctctgctgcccgggctgcgccagagccgcggacgggcgcgcagagcgccggggactccggagccgatccctagcgccgcgatgcggagcacctactgcaggagatcgggggcctgggacgcgctggccgaggtgtgatcggaccccaggctagccacaaagggcacttggccccagggctaggagagcgaggggagagcacagccacccgcctcggcggcccgggactcggctcgactcgccggagaatgcgcccgaggacgacggggcgccagagccgcggtgctttcaactggcgagcgcgaatgggggtgcactggagtaaggcagagtgatgcgggggggcaactcgcctggcaccgagatcgccgccgtgcccttccctggacccggcgtcgcccaggatggctgccccgagccatgggccgcggcggagctagcgcggagcgcccgaccctcgacccccgagtcccggagccggccccgcgcggggccacgcgtccctcgggcgctggttcctaaggaggacgacagcaccagcttctcctttctcccttcccttccctgccccgcactcctccccctgctcgctgttgttgtgtgtcagcacttggctggggacttcttgaacttgcagggagaataacttgcgcaccccactttgcgccggtgcctttgccccagcggagcctgcttcgccatctccgagccccaccgcccctccactcctcggccttgcccgacactgagacgctgttcccagcgtgaaaagagagactgcgcggccggcacccgggagaaggaggaggcaaagaaaaggaacggacattcggtccttgcgccaggtcctttgaccagagtttttccatgtggacgctctttcaatggacgtgtccccgcgtgcttcttagacggactgcggtctcctaaaggtcgaccatggtggccgggacccgctgtcttctagcgttgctgcttccccaggtcctcctgggcggcgcggctggcctcgttccggagctgggccgcaggaagttcgcggcggcgtcgtcgggccgcccctcatcccagccctctgacgaggtcctgagcgagttcgagttgcggctgctcagcatgttcggcctgaaacagagacccacccccagcagggacgccgtggtgcccccctacatgctagacctgtatcgcaggcactcaggtcagccgggctcacccgccccagaccaccggttggagagggcagccagccgagccaacactgtgcgcagcttccaccatgaagaatctttggaagaactaccagaaacgagtgggaaaacaacccggagattcttctttaatttaagttctatccccacggaggagtttatcacctcagcagagcttcaggttttccgagaacagatgcaagatgctttaggaaacaatagcagtttccatcaccgaattaatatttatgaaatcataaaacctgcaacagccaactcgaaattccccgtgaccagacttttggacaccaggttggtgaatcagaatgcaagcaggtgggaaagttttgatgtcacccccgctgtgatgcggtggactgcacagggacacgccaaccatggattcgtggtggaagtggcccacttggaggagaaacaaggtgtctccaagagacatgttaggataagcaggtctttgcaccaagatgaacacagctggtcacagataaggccattgctagtaacttttggccatgatggaaaagggcatcctctccacaaaagagaaaaacgtcaagccaaacacaaacagcggaaacgccttaagtccagctgtaagagacaccctttgtacgtggacttcagtgacgtggggtggaatgactggattgtggctcccccggggtatcacgccttttactgccacggagaatgcccttttcctctggctgatcatctgaactccactaatcatgccattgttcagacgttggtcaactctgttaactctaagattcctaaggcatgctgtgtcccgacagaactcagtgctatctcgatgctgtaccttgacgagaatgaaaaggttgtattaaagaactatcaggacatggttgtggagggttgtgggtgtcgctagtacagcaaaattaaatacataaatatatatatatatatatattttagaaaaaagaaaaaaacaaacaaacaaaaaaaccccaccccagttgacactttaatatttcccaatgaagactttatttatggaatggaatggaaaaaaaaacagctattttgaaaatatatttatatctacgaaaagaagttgggaaaacaaatattttaatcagagaattattccttaaagatttaaaatgtatttagttgtacattttatatgggttcaaccccagcacatgaagtataatggtcagatttattttgtatttatttactattataaccactttttaggaaaaaaatagctaatttgtatttatatgtaatcaaaagaagtatcgggtttgtacataattttccaaaaattgtagttgttttcagttgtgtgtatttaagatgaaaagtctacatggaaggttactctggcaaagtgcttagcacgtttgcttttttgcagtgctactgttgagttcacaagttcaagtccagaaaaaaaaagtggataatccactctgctgactttcaagattattatattattcaattctcaggaatgttgcagagtgattgtccaatccatgagaatttacatccttattaggtggaatatttggataagaaccagacattgctgatctattatagaaactctcctcctgccccttaatttacagaaagaataaagcaggatccatagaaataattaggaaaacgatgaacctgcaggaaagtgaatgatggtttgttgttcttctttcctaaattagtgatcccttcaaaggggctgatctggccaaagtattcaataaaacgtaagatttcttcattattgatattgtggtcatatatatttaaaattgatatctcgtggccctcatcaagggttggaaatttatttgtgttttacctttacctcatctgagagctctttattctccaaagaacccagttttctaactttttgcccaacacgcagcaaaattatgcacatcgtgttttctgcccaccctctgttctctgacctatcagcttgcttttctttccaaggttgtgtgtttgaacacatttctccaaatgttaaacctatttcagataataaatatcaaatctctggca

SEQ ID NO: 13 - protein, 396 aa, Homo sapiens
MVAGTRCLLALLLPQVLLGGAAGLVPELGRRKFAAASSGRPSSQPSDEVLSEFELRLLSMFGLKQRPTPSRDAVVPPYMLDLYRRHSGQPGSPAPDHRLERAASRANTVRSFHHEESLEELPETSGKTTRRFFFNLSSIPTEEFITSAELQVFREQMQDALGNNSSFHHRINIYEIIKPATANSKFPVTRLLDTRLVNQNASRWESFDVTPAVMRWTAQGHANHGFVVEVAHLEEKQGVSKRHVRISRSLHQDEHSWSQIRPLLVTFGHDGKGHPLHKREKRQAKHKQRKRLKSSCKRHPLYVDFSDVGWNDWIVAPPGYHAFYCHGECPFPLADHLNSTNHAIVQTLVNSVNSKIPKACCVPTELSAISMLYLDENEKVVLKNYQDMVVEGCGCR

SEQ ID NO: 14 - protein, 116 aa, Homo sapiens
SPKHHSQRARKKNKNCRRHSLYVDFSDVGWNDWIVAPPGYQAFYCHGDCPFPLADHLNSTNHAIVQTLVNSVNSSIPKACCVPTELSAISMLYLDEYDKVVLKNYQEMVVEGCGCR

SEQ ID NO: 15 - protein, 132 aa, Homo sapiens
NQNRNKSSSHQDSSRMSSVGDYNTSEQKQACKKHELYVSFRDLGWQDWIIAPEGYAAFYCDGECSFPLNAHMNATNHAIVQTLVHLMFPDHVPKPCCAPTKLNAISVLYFDDSSNVILKKYRNMVVRSCGCH

SEQ ID NO: 16 - protein, 132 aa, Homo sapiens
QQSRNRSTQSQDVARVSSASDYNSSELKTACRKHELYVSFQDLGWQDWIIAPKGYAANYCDGECSFPLNAHMNATNHAIVQTLVHLMNPEYVPKPCCAPTKLNAISVLYFDDNSNVILKKYRNMVVRACGCH

SEQ ID NO: 17 - protein, 139 aa, Homo sapiens
STGSKQRSQNRSKTPKNQEALRMANVAENSSSDQRQACKKHELYVSFRDLGWQDWIIAPEGYAAYYCEGECAFPLNSYMNATNHAIVQTLVHFINPETVPKPCCAPTQLNAISVLYFDDSSNVILKKYRNMVVRACGCH

SEQ ID NO: 18 - protein, 139 aa, Homo sapiens
AVRPLRRRQPKKSNELPQANRLPGIFDDVHGSHGRQVCRRHELYVSFQDLGWLDWVIAPQGYSAYYCEGECSFPLDSCMNATNHAILQSLVHLMKPNAVPKACCAPTKLSATSVLYYDSSNNVILRKHRNMVVKACGCH

SEQ ID NO: 19 - protein, 120 aa, Homo sapiens
APLATRQGKRPSKNLKARCSRKALHVNFKDMGWDDWIIAPLEYEAFHCEGLCEFPLRSHLEPTNHAVIQTLMNSMDPESTPPTCCVPTRLSPISILFIDSANNVVYKQYEDMVVESCGCR

SEQ ID NO: 20 - protein, 120 aa, Mus musculus
TAFASRHGKRHGKKSRLRCSRKPLHVNFKELGWDDWIIAPLEYEAYHCEGVCDFPLRSHLEPTNHAIIQTLMNSMDPGSTPPSCCVPTKLTPISILYIDAGNNVVYKQYEDMVVESCGCR

SEQ ID NO: 21 - protein, 146 aa, Mus musculus
TALAGTRGAQGSGGGGGGGGGGGGGGGGGGGGAGRGHGRRGRSRCSRKSLHVDFKELGWDDWIIAPLDYEAYHCEGVCDFPLRSHLEPTNHAIIQTLLNSMAPDAAPASCCVPARLSPISILYIDAANNVVYKQYEDMVVEACGCR

SEQ ID NO: 22 - protein, 108 aa, Homo sapiens
NAKGNYCKRTPLYIDFKEIGWDSWIIAPPGYEAYECRGVCNYPLAEHLTPTKHAIIQALVHLKNSQKASKACCVPTKLEPISILYLDKGVVTYKFKYEGMAVSECGCR

SEQ ID NO: 23 - protein, 110 aa, Homo sapiens
SAGAGSHCQKTSLRVNFEDIGWDSWIIAPKEYEAYECKGGCFFPLADDVTPTKHAIVQTLVHLKFPTKVGKACCVPTKLSPISVLYKDDMGVPTLKYHYEGMSVAECGCR

SEQ ID NO: 24 - protein, 396 aa, synthetic construct
  source 1..396: note = L51P
MVAGTRCLLALLLPQVLLGGAAGLVPELGRRKFAAASSGRPSSQPSDEVPSEFELRLLSMFGLKQRPTPSRDAVVPPYMLDLYRRHSGQPGSPAPDHRLERAASRANTVRSFHHEESLEELPETSGKTTRRFFFNLSSIPTEEFITSAELQVFREQMQDALGNNSSFHHRINIYEIIKPATANSKFPVTRLLDTRLVNQNASRWESFDVTPAVMRWTAQGHANHGFVVEVAHLEEKQGVSKRHVRISRSLHQDEHSWSQIRPLLVTFGHDGKGHPLHKREKRQAKHKQRKRLKSSCKRHPLYVDFSDVGWNDWIVAPPGYHAFYCHGECPFPLADHLNSTNHAIVQTLVNSVNSKIPKACCVPTELSAISMLYLDENEKVVLKNYQDMVVEGCGCR